European Patent Specification EP 3 229 612 B1, published June 26, 2024. Title: FLAVOR COMPOSITIONS AND PET FOOD PRODUCTS CONTAINING THE SAME. Applicant: MARS, INCORPORATED. The sequence listing filed with the application follows.

SEQUENCE LISTING (4 sequences)

SEQ ID NO: 1 - DNA, 2526 bp, Felis catus
atgtcactcccggcggctcacctggtcggcctgcagctctccctctcctgctgctgggctctcagctgccacagcacagagacgtctgccgacttcagcctccctggggattacctcctcgcaggtctgttccctctgcactctgactgtccgggcgtgaggcaccggcccacggtgaccctctgtgacaggcccgacagcttcaacggtcacggctaccacctcttccaggccatgcggtttggcatcgaggagataaacaactccacggccctcctgccgaacgtcaccctgggataccagctgtacgacgtgtgctcggagtctgccaacgtgtatgccacactaaacgtgctctccctgctggggacacatcacgtagagatccgagcagacccttcccactattcgcccgccgccctggctgtcattgggcctgacaccaccaaccacgcagccaccactgcagccctgctgagccccttcctggtgcccctgatcagctacgaggccagcagcgtgacgctcggagtgaagcggcattacccctcgtttctgcgcaccatccccagcgacaagcaccaggtggaggccatggtgctgctgctgcagagcttcgggtgggtctggatctcggtggtcggcagcgacggcgactacgggcagctgggggtgcaggcgctggaggagcaggccacccagcagggcatctgcgttgccttcaaggacatcatccccttctctgcccggccgggcgacgagaggatgcagggcatcatgcaccacctggcccgagcgaggaccaccgttgtggtcgttttctccagcaggcagctggccagggtgttctttgagtcggtggtgctggccaacctgactgccaaggtgtggatcgcctcagaagactgggccatctctagacacatcagcaatgtgcccgggatccagggcattggcacagtgctgggtgtggccatccagcagaggcttgtccctggcctgaaggagtttgaagaggcctatgtccaggcagataagggggcccctgggccttgctccaggacctccgagtgcagcagcaaccagctctgtagagagtgtcgggctttcacggcagagcagatgcccacgctcggggcattctccatgagctctgcttataacgcctaccgggcagtctacgcagtggcccatggcctccaccagctcctgggctgtgcctctggagcctgttccagggaccgagtctacccctggcagcttctggagcagatccgcaaggtgaatttcctcctacacaaggacaccgtgaggtttaatgacaacggggaccctctcagtggctacgacataattgcctgggactggagtggccccaagtggaacttcagggtcattggctcctccatgtggcctccagttcagctggacataaataaaaccaaaatccggtggcacgggaaggacaaccaggtgccaaagtctgtgtgctccagcgactgcctcgaagggcaccagcgagtgatttcgggtttctaccactgttgctttgagtgtgtgccctgtgaggccgggagcttcctcaacaagagcgacctccacagctgccagccttgtgggaaagaagagtgggcacccgcgggaagtgaaacctgctttccacgcaccgtggtgtttttgacttggcacgagaccatctcttgggtgctgctggcagctaatacgttgctgctgctgctggtgactgggactgctggcctgtttgcctggcacttagacacccctgtggtgaagtccgctgggggccgactgtgcttcttcatgctgggctccctggcagggggcagctgtgggctctacggcttttttggggagcccacgctgcccacatgcttgttgcgccaaagcctccttgccctgggttttgccatcttcctgtcctgcctgaccatccgctccttccaactggtcttcatcttcaagttttctgccaaggtacccaccttctaccgtgcctgggtccaaaaccacggtcctggcctatttgtggtgatcagctcaatggcccagctgctcatctgtctaacttggctggcggtgtggaccccactgcccaccagggagtaccagcgcttccctcagctggtggtgcttgattgcacagaggccaactcaccgggcttcatgttggctttcgcctacaatggcctcctgtccgtcagcgcctttgcctgcagctacctgggcaaggacctgccagagaactacaacgaggccaaatgtgtcacttttagtctgctgctcaacttcgtgtcctggattgccttcttcaccacggccagcgtctaccagggcaagtacttgcccgcggtcaacgtgctggcggcgctgagcagcctgagtggcggcttcagcggttatttcctccccaagtgctacgtgatcctgtgccgcccagatctcaacagcacagagcacttccaggcctccatccaggagtacacgaggcgctgcggctccacctga

SEQ ID NO: 2 - protein, 841 aa, Felis catus
MSLPAAHLVGLQLSLSCCWALSCHSTETSADFSLPGDYLLAGLFPLHSDCPGVRHRPTVTLCDRPDSFNGHGYHLFQAMRFGIEEINNSTALLPNVTLGYQLYDVCSESANVYATLNVLSLLGTHHVEIRADPSHYSPAALAVIGPDTTNHAATTAALLSPFLVPLISYEASSVTLGVKRHYPSFLRTIPSDKHQVEAMVLLLQSFGWVWISVVGSDGDYGQLGVQALEEQATQQGICVAFKDIIPFSARPGDERMQGIMHHLARARTTVVVVFSSRQLARVFFESVVLANLTAKVWIASEDWAISRHISNVPGIQGIGTVLGVAIQQRLVPGLKEFEEAYVQADKGAPGPCSRTSECSSNQLCRECRAFTAEQMPTLGAFSMSSAYNAYRAVYAVAHGLHQLLGCASGACSRDRVYPWQLLEQIRKVNFLLHKDTVRFNDNGDPLSGYDIIAWDWSGPKWNFRVIGSSMWPPVQLDINKTKIRWHGKDNQVPKSVCSSDCLEGHQRVISGFYHCCFECVPCEAGSFLNKSDLHSCQPCGKEEWAPAGSETCFPRTVVFLTWHETISWVLLAANTLLLLLVTGTAGLFAWHLDTPVVKSAGGRLCFFMLGSLAGGSCGLYGFFGEPTLPTCLLRQSLLALGFAIFLSCLTIRSFQLVFIFKFSAKVPTFYRAWVQNHGPGLFVVISSMAQLLICLTWLAVWTPLPTREYQRFPQLVVLDCTEANSPGFMLAFAYNGLLSVSAFACSYLGKDLPENYNEAKCVTFSLLLNFVSWIAFFTTASVYQGKYLPAVNVLAALSSLSGGFSGYFLPKCYVILCRPDLNSTEHFQASIQEYTRRCGST

SEQ ID NO: 3 - DNA, 2597 bp, Felis catus
atgcccggcctcgctctcctgggcctcacggctctcctgggcctcacggctccttggaccacggggagggcgcaacgtcctgcttgtcacagcagctcaggatgcagggggactatgtgctgggtgggctcttccctctgggctctgccgagggtacaggtcttggcgacgggctgcagcccaatgccaccgtgtgcaccaggttctcgtctctgggcctgctctgggcgctggccgtgaagatggcggtggaggagatcaacaacgggtcggccctgctgcccgggctgcacctgggctatgacctctttgacacgtgttcagagcccatggtggccatgaagcccagcctcgtgttcatggccaaagcaggcagctgcagcattgccgcctactgcaattacacacagtaccagccccgcgtgctggccgtcatcgggccccactcgtctgagctcgccctcgtcaccggcaagttcttcagcttcttccttgtgcctcaggtcagctacggcgccagcaccgaccggctgagcaaccgggagatcttcccgtccttcttccgcacggtgcccagcgaccaggtgcaggtggcggccatggtggagctgctgcaggagctcggctggaactgggtggcggcggtgggtagtgacgacgagtatggccggcagggcctgagcctcttctccggcctggccagcgccaggggcatctgcatcgcgcatgagggcctggtgccactgccgccaggcagcctgcggctgggcgccctacagggcctgctgcgccaggtgaaccagagcagcgtgcaggtggtggtgctgttctcctccgcccacgcggcccgcaccctcttcagctacagcatccgctgcaagctctcacccaaggtgtgggtggccagcgaggcctggctgacctcagacctggtcatgacgctgcccggcatgcctggggtgggcaccgtgctgggcttcctgcagcagggcgccccgatgccggagttcccatcctacgtgcggacccgcctggccctggccgctgaccctgccttctgcgcctcgctggacgctgaacagccaggcctggaggagcacgtggtggggccacgctgcccccaatgtgaccacgtcacgctagagaacctatctgcggggctgctgcaccaccagaccttcgctgcctacgcggctgtgtatggcgtggcccaggcccttcacaacacactgcgctgcaatgcctcgggctgccccaggcgggagcctgtgcggccctggcagctcctagagaacatgtacaacgtgagcttccgtgctcgcggcctggcactgcagttcgacgccagcgggaacgtgaacgtggattacgacctgaaactgtgggtgtggcaggacccgacgcccgagctgcgcaccgtaggcaccttcaagggccgcctggagctctggcgctctcagatgtgctggcacacgccggggaagcagcagcccgtgtcccagtgctcccggcagtgcaaggagggccaggtgcgccgcgtgaagggcttccactcttgctgttacgactgcgtggactgcaaggcgggcagttatcagcgcaacccagatgacctcctctgcacccagtgtgaccaggaccagtggtccccagaccggagcacacgctgcttcgcccgcaagcccatgttcctggcatggggggagccagctgtgctgctactgctcgcgctgctggctctggcgctgggcctggcgctggcagccctggggctcttcctctggcactcggacagcccgctggttcaggcctcaggtgggccacgggcctgctttggcctggcctgcctgggcctggtctgcctcagtgtcctcctgttccctggccagccaggccctgccagctgcctggcccagcagccactgttccacctcccactcactggctgcctgagcacgcttttcctgcaagcggccgagatatttgtggggtcggagctgccaccaagctgggctgagaagatgcgtggccgcctgcgggggccctgggcctggctggtggtgctgcttgctatgctggcagaagccgcattgtgtgcctggtacctggtagccttcccgccagaggtggtgacggactggcgggtactgcccacagaggcgctggtgcactgccacgtgcactcctggatcagcttcggcctggtgcatgccactaacgccatgctggccttcctctgcttcctgggcactttcctggtgcagagccggccaggccgctacaatggtgcccgcggcctcacctttgccatgctggcctacttcatcacctggatctcctttgtgcccctctttgccaatgtgcacgtggcctaccagcctgccgtgcagatgggcaccatcctcctctgtgccctgggtatcctagccaccttccacctgcccaagtgctacctgctgctgcagcggccggagctcaacacccctgagttcttcctggaagacaatgccagagcacagggcagcagttgggggcaggggaggggagaatcggggcaaaaacaagtgacacccgatccagtgacctcaccgcagtga

SEQ ID NO: 4 - protein, 865 aa, Felis catus
MPGLALLGLTALLGLTALLDHGEGATSCLSQQLRMQGDYVLGGLFPLGSAEGTGLGDGLQPNATVCTRFSSLGLLWALAVKMAVEEINNGSALLPGLHLGYDLFDTCSEPMVAMKPSLVFMAKAGSCSIAAYCNYTQYQPRVLAVIGPHSSELALVTGKFFSFFLVPQVSYGASTDRLSNREIFPSFFRTVPSDQVQVAAMVELLQELGWNWVAAVGSDDEYGRQGLSLFSGLASARGICIAHEGLVPLPPGSLRLGALQGLLRQVNQSSVQVVVLFSSAHAARTLFSYSIRCKLSPKVWVASEAWLTSDLVMTLPGMPGVGTVLGFLQQGAPMPEFPSYVRTRLALAADPAFCASLDAEQPGLEEHVVGPRCPQCDHVTLENLSAGLLHHQTFAAYAAVYGVAQALHNTLRCNASGCPRREPVRPWQLLENMYNVSFRARGLALQFDASGNVNVDYDLKLWVWQDPTPELRTVGTFKGRLELWRSQMCWHTPGKQQPVSQCSRQCKEGQVRRVKGFHSCCYDCVDCKAGSYQRNPDDLLCTQCDQDQWSPDRSTRCFARKPMFLAWGEPAVLLLLALLALALGLALAALGLFLWHSDSPLVQASGGPRACFGLACLGLVCLSVLLFPGQPGPASCLAQQPLFHLPLTGCLSTLFLQAAEIFVGSELPPSWAEKMRGRLRGPWAWLVVLLAMLAEAALCAWYLVAFPPEVVTDWRVLPTEALVHCHVHSWISFGLVHATNAMLAFLCFLGTFLVQSRPGRYNGARGLTFAMLAYFITWISFVPLFANVHVAYQPAVQMGTILLCALGILATFHLPKCYLLLQRPELNTPEFFLEDNARAQGSSWGQGRGESGQKQVTPDPVTSPQ